European Patent Application EP 4 692 336 A1, published February 11, 2026. Title: PURIFICATION OF BIONANOPARTICLES. Applicant: ArcticZymes AS. Application EP, filed August 8, 2024. The sequence listing filed with the application follows.

SEQUENCE LISTING (68 sequences)

SEQ ID NO: 1 - protein, 211 aa, Vibrio cholerae
APISFSHAKNEAVKIYRDHPVSFYCGCEIRWQGKKGIPDLESCGYQVRKNENRASRIEWEHVVPAWQFGHQLQCWQQGGRKNCTRTSPEFNQMEADLHNLTPAIGEVNGNRSNFSFSQWNGIDGVTYGQCEMQVNFKERTAMPPERARGAIARTYLYMSEQYGLRLSKAQNQLMQAWNNQYPVSEWECVRDQKIEKVQGNSNRFVREQCPN

SEQ ID NO: 2 - protein, 211 aa, synthetic construct
  VARIANT 22: note = x at position 22 is S, D or E
APISFSHAKNEAVKIYRDHPVXFYCGCEIRWQGKKGIPDLESCGYQVRKNENRASRIEWEHVVPAWQFGHQLQCWQQGGRKNCTRTSPEFNQMEADLHNLTPAIGEVNGNRSNFSFSQWNGIDGVTYGQCEMQVNFKERTAMPPERARGAIARTYLYMSEQYGLRLSKAQNQLMQAWNNQYPVSEWECVRDQKIEKVQGNSNRFVREQCPN

SEQ ID NO: 3 - protein, 231 aa, Vibrio cholerae
MMIFRFVTTLAASLPLLTFAAPISFSHAKNEAVKIYRDHPVSFYCGCEIRWQGKKGIPDLESCGYQVRKNENRASRIEWEHVVPAWQFGHQLQCWQQGGRKNCTRTSPEFNQMEADLHNLTPAIGEVNGNRSNFSFSQWNGIDGVTYGQCEMQVNFKERTAMPPERARGAIARTYLYMSEQYGLRLSKAQNQLMQAWNNQYPVSEWECVRDQKIEKVQGNSNRFVREQCPN

SEQ ID NO: 4 - protein, 213 aa, synthetic construct
  VARIANT 1..213: note = Wherein X is S, D or E
APPSSFSKAKKEAVKIYLDYPTXFYCGCDITWKNKKKGIPELESCGYQVRKQEKRASRIEWEHVVPAWQFGHQRQCWQKGGRKNCTRNDKQFKSMEADLHNLVPAIGEVNGDRSNFRFSQWNGSKGAFYGQCAFKVDFKGRVAEPPAQSRGAIARTYLYMNNEYKFNLSKAQRQLMEAWNKQYPVSTWECTRDERIAKIQGNHNQFVYKACTK

SEQ ID NO: 5 - protein, 213 aa, Allivibrio salmonicidae
APPSSFSKAKKEAVKIYLDYPTSFYCGCDITWKNKKKGIPELESCGYQVRKQEKRASRIEWEHVVPAWQFGHQRQCWQKGGRKNCTRNDKQFKSMEADLHNLVPAIGEVNGDRSNFRFSQWNGSKGAFYGQCAFKVDFKGRVAEPPAQSRGAIARTYLYMNNEYKFNLSKAQRQLMEAWNKQYPVSTWECTRDERIAKIQGNHNQFVYKACTK

SEQ ID NO: 6 - protein, 234 aa, Allivibrio salmonicidae
MKLIRLVISLIAVSFTVNVMAAPPSSFSKAKKEAVKIYLDYPTSFYCGCDITWKNKKKGIPELESCGYQVRKQEKRASRIEWEHVVPAWQFGHQRQCWQKGGRKNCTRNDKQFKSMEADLHNLVPAIGEVNGDRSNFRFSQWNGSKGAFYGQCAFKVDFKGRVAEPPAQSRGAIARTYLYMNNEYKFNLSKAQRQLMEAWNKQYPVSTWECTRDERIAKIQGNHNQFVYKACTK

SEQ ID NO: 7 - protein, 213 aa, Vibrio vulnificus
APPSSFSAAKQQAVKIYQDHPISFYCGCDIEWQGKKGIPNLETCGYQVRKQQTRASRIEWEAVVPAWQFGHHRQCWQKGGRKNCSKNDQQFRLMEADLHNLTPAIGEVNGDRSNFNFSQWNGVDGVSYGRCEMQVNFKQRKVMPPDRARGSIARTYLYMSQEYGFQLSKQQQQLMQAWNKSYPVDEWECTRDDRIAKIQGNHNPFVQQSCQTQ

SEQ ID NO: 8 - protein, 245 aa, Serratia marcescens
DTLESIDNCAVGCPTGGSSNVSIVRHAYTLNNNSTTKFANWVAYHITKDTPASGKTRNWKTDPALNPADTLAPADYTGANAALKVDRGHQAPLASLAGVSDWESLNYLSNITPQKSDLNQGAWARLEDQERKLIDRADISSVYTVTGPLYERDMGKLPGTQKAHTIPSAYWKVIFINNSPAVNHYAAFLFDQNTPKGADFCQFRVTVDEIEKRTGLIIWAGLPDDVQASLKSKPGVLPELMGCKN

SEQ ID NO: 9 - protein, 245 aa, synthetic construct
  VARIANT 51: note = Wherein X at position 51 is P, L, G, A, V, or I
  VARIANT 52: note = Wherein X at position 52 is A, R, H, or K
  VARIANT 53: note = Wherein X at position 53 is S, R, H, or K
  VARIANT 54: note = Wherein X at position 54 is G, R, H, or K
  VARIANT 56: note = Wherein X at position 56 is T, R, H, or K
  VARIANT 58: note = Wherein X at position 58 is N, R, H, or K
  VARIANT 73: note = Wherein X at position 73 is P, R, H, or K
  VARIANT 74: note = Wherein X at position 74 is A, R, H, or K
  VARIANT 77: note = Wherein X at position 77 is T, R, H, or K
  VARIANT 78: note = Wherein X at position 78 is G, R, H, or K
  VARIANT 80: note = Wherein X at position 80 is N, R, H, or K
  VARIANT 81: note = Wherein X at position 81 is A, R, H, or K
  VARIANT 119: note = Wherein X at position 119 is N, R, H, or K
  VARIANT 120: note = Wherein X at position 120 is Q, R, H, or K
  VARIANT 124: note = Wherein X at position 124 is A, R, H, or K
  VARIANT 195: note = Wherein X at position 195 is P, R, H, or K
DTLESIDNCAVGCPTGGSSNVSIVRHAYTLNNNSTTKFANWVAYHITKDTXXXXKXRXWKTDPALNPADTLAXXDYXXAXXALKVDRGHQAPLASLAGVSDWESLNYLSNITPQKSDLXXGAWXRLEDQERKLIDRADISSVYTVTGPLYERDMGKLPGTQKAHTIPSAYWKVIFINNSPAVNHYAAFLFDQNTXKGADFCQFRVTVDEIEKRTGLIIWAGLPDDVQASLKSKPGVLPELMGCKN

SEQ ID NO: 10 - protein, 245 aa, synthetic construct
DTLESIDNCAVGCPTGGSSNVSIVRHAYTLNNNSTTKFANWVAYHITKDTLASGKTRNWKTDPALNPADTLAPADYRGANAALKVDRGHQAPLASLAGVSDWESLNYLSNITPQKSDLNQGAWRRLEDQERKLIDRADISSVYTVTGPLYERDMGKLPGTQKAHTIPSAYWKVIFINNSPAVNHYAAFLFDQNTPKGADFCQFRVTVDEIEKRTGLIIWAGLPDDVQASLKSKPGVLPELMGCKN

SEQ ID NO: 11 - protein, 245 aa, synthetic construct
DTLESIDNCAVGCPTGGSSNVSIVRHAYTLNNNSTTKFANWVAYHITKDTLRSRKTRNWKTDPALNPADTLARRDYRRANRALKVDRGHQAPLASLAGVSDWESLNYLSNITPQKSDLNQGAWRRLEDQERKLIDRADISSVYTVTGPLYERDMGKLPGTQKAHTIPSAYWKVIFINNSPAVNHYAAFLFDQNTRKGADFCQFRVTVDEIEKRTGLIIWAGLPDDVQASLKSKPGVLPELMGCKN

SEQ ID NO: 12 - protein, 228 aa, Photobacterium profundum
APPSSFSKAKRLAVEIYQDHPTSFYCGCAITWQGKKGLPDLASCGYEVRKQEKRANRIEWEHVVPAENFGRAFVEWREGHPQCVNSKGKAYKGRSCATKMNPTYRSMQADLHNLTPAVGEVNGDRSNYAFLPWNGNNGAFYGQCDMKIDFKNRRADPPEQSRGAIARTYLYMNQEYKMALSSQQRQLMEAWNRQYPISTWECERDRRIANIQDNHNSFVLQACKKAGY

SEQ ID NO: 13 - protein, 211 aa, synthetic construct
APISFSHAKNEAVKIYRDHPVSFYCGCEIRWQGKKGIPDLESCGYQVRKQENRASRIEWEHVVPAWQFGHQLQCWQQGGRKNCTRTSPEFNQMEADLHNLTPAIGEVNGNRSNFSFSQWNGIDGVTYGQCEMQVNFKERTAMPPERARGAIARTYLYMSEQYGLRLSKAQNQLMQAWNNQYPVSEWECVRDQKIEKVQGNSNRFVREQCPN

SEQ ID NO: 14 - protein, 211 aa, synthetic construct
APISFSHAKNEAVKIYRDHPVSFYCGCEIRWQGKKGIPDLESCGYQVRKNEKRASRIEWEHVVPAWQFGHQLQCWQQGGRKNCTRTSPEFNQMEADLHNLTPAIGEVNGNRSNFSFSQWNGIDGVTYGQCEMQVNFKERTAMPPERARGAIARTYLYMSEQYGLRLSKAQNQLMQAWNNQYPVSEWECVRDQKIEKVQGNSNRFVREQCPN

SEQ ID NO: 15 - protein, 211 aa, synthetic construct
APISFSHAKNEAVKIYRDHPVSFYCGCEIRWQGKKGIPDLESCGYQVRKQEKRASRIEWEHVVPAWQFGHQLQCWQQGGRKNCTRTSPEFNQMEADLHNLTPAIGEVNGNRSNFSFSQWNGIDGVTYGQCEMQVNFKERTAMPPERARGAIARTYLYMSEQYGLRLSKAQNQLMQAWNNQYPVSEWECVRDQKIEKVQGNSNRFVREQCPN

SEQ ID NO: 16 - protein, 211 aa, Vibrio cholerae
APISFSHAKNEAVKIYRDHPVSFYCGCEIRWQGKKGIPDLESCGYQVRKNENRASRIEWEHVVPAWQFGHQLQCWQQGGRKNCTRTSPEFNQMEADLHNLTPAIGEVNGDRSNFSFSQWNGVDGVTYGQCEMQVNFKERTAMPPERARGAIARTYLYMSEQYGLRLSKAQSQLMQAWNNQYPVSEWECVRDQRIEKVQGNSNRFVREQCPN

SEQ ID NO: 17 - protein, 211 aa, Vibrio cholerae
APISFSHAKNEAVKIYRDHPVSFYCGCEIRWQGKKGIPDLESCGYQVRKNENRASRIEWEHVVPAWQFGHQLQCWQQGGRKNCTRTSPEFNQMEADLHNLTPAIGEVNGDRSNFSFSQWNGIDGVTYGQCEMQVNFKERTAMPPERARGAIARTYLYMSEQYGLRLSKAQNQLMQAWNNQYPVSEWECVRDQKIEKVQGNSNRFVREQCPN

SEQ ID NO: 18 - protein, 211 aa, Vibrio cholerae
APMSFSHAKNEAVKIYRDHPVSFYCGCEIRWQGKKGIPDLESCGYQVRKNENRASRIEWEHVVPAWQFGHQLQCWQQGGRKNCTRTSPEFNQMEADLHNLTPAIGEVNGDRSNFSFSQWNGIDGVTYGQCEMQVNFKERTAMPPERARGAIARTYLYMSEQYGLRLSKAQNQLMQAWNNQYPVSEWECVRDQKIEKVQGNSNRFVREQCPN

SEQ ID NO: 19 - protein, 211 aa, Vibrio cholerae
APISFSHAKNEAVKIYRDHPVSFYCGCEIRWQGKKGIPDLESCGYQVRKNENRASRIEWEHVMPAWQFGHQLQCWQQGGRKNCTRTSPEFNQMEADLHNLTPAIGEVNGDRSNFSFSQWNGIDGVTYGQCEMQVNFKERTAMPPERARGAIARTYLYMSEQYGLRLSKAQNQLMQAWNNQYPVSEWECVRDQKIEKVQGNSNRFVREQCPN

SEQ ID NO: 20 - protein, 211 aa, Vibrio cholerae
APISFSHAKNEAVKIYRDHPVSFYCGCEIRWQGKKGIPDLESCGYQVRKNENRASRIEWEHVVPAWQFGHQLQCWQQGGRKNCTRTSPEFNQMEADLHNLTPAIGEVNGDRSNFSFSQWNGIDGVTYGQCEMQVNFKERTAMPPERARGAIARTYLYMSEQYGLRLSKAQNQLMQAWNNQYPVSEWECVRDQRIEKVQGNSNRFVREQCPN

SEQ ID NO: 21 - protein, 213 aa, synthetic construct
APPSSFSKAKKEAVKIYLDYPTSFYCGCDITWKNKKKGIPELESCGYEVRKQEKRASRIEWEHVVPAWQFGHQRQCWQKGGRKNCTRNDKQFKSMEADLHNLVPAIGEVNGDRSNFRFEQWDGSKGAFYGQCAFKVDFKGRVAEPPAQSRGAIARTYLYMNNEYKFNLSKAQRQLMEAWNKQYPVSTWECTRDERIAKIQENHNQFVYKACTK

SEQ ID NO: 22 - protein, 213 aa, synthetic construct
APPSSFSKAKKEAVKIYLDYPTSFYCGCDITWKNKKKGIPELESCEYEVRKQEKRASRIEWEHVVPAWQFGHQRQCWQKGGRKNCTRNDKQFKSMEADLHNLVPAIGEVNGDRSNFRFEQWDGDKGADYGQCAFKVDFKGRVAEPPADSRGAIARTYLYMNNEYKFELSKAQRQLMEAWNKQYPVSTWECTRDERIAKIQENHNQFVYKACTK

SEQ ID NO: 23 - protein, 213 aa, synthetic construct
APPSSFSKAKKEAVKIYLDYPTSFYCGCDITWKNKKKGIPELESCKYQVRKQEKRASRIEWEHVVPAWQFGHQRQCWQKGGRKNCTRNDKQFKSMEADLHNLVPAIGEVNGDRSNFRFSQWKGSKGAFYGKCAFKVDFKGRVAEPPAQSRGAIARTYLYMNNEYKFNLSKAQRQLMEAWNKQYPVSTWECTRDERIAKIQKNHNQFVYKACTK

SEQ ID NO: 24 - protein, 213 aa, synthetic construct
APPSSFSKAKKEAVKIYLDYPESFYCGCDITWKNKKKGIPELESCGYQVRKQEKRASRIEWEHVVPAWQFGHQRQCWQKGGRKNCTRNDKQFKSMEADLHNLVPAIGEVNGDRSNFRFSQWNGSKGAFYGQCAFKVDFKGRVAEPPAQSRGAIARTYLYMNNEYKFNLSKAQRQLMEAWNKQYPVSTWECTRDERIAKIQGNHNQFVYKACTK

SEQ ID NO: 25 - protein, 213 aa, synthetic construct
APPSSFSKAKKEAVKIYLDYPTSFYCGCDITWKNKKKGIPELESCGYQVRKQEKRASRIEWEHVVPAWQFGHQRQCWQKGGRKNCTRNDKQFKSMEADLHNLVPAIGEVNGDRSNERFSQWNGSKGAFYGQCAFKVDFKGRVAEPPAQSRGAIARTYLYMNNEYKFNLSKAQRQLMEAWNKQYPVSTWECTRDERIAKIQGNHNQFVYKACTK

SEQ ID NO: 26 - protein, 213 aa, synthetic construct
APPSSFSKAKKEAVKIYLDYPTSFYCGCDITWKNKKKGIPELESCGYQVRKQEKRASRIEWEHVVPADQFGHQRQCWQKGGRKNCTRNDKQFKSMEADLHNLVPAIGEVNGDRSRFRFSQWNGSKGAFYGQCAFKVDFKGRVAEPPAQSRGAIARTYLYMNNEYKFNLSKAQRQLMEAWNKQYPVSTWECTRDERIAKIQGNHNQFVYKACTK

SEQ ID NO: 27 - protein, 213 aa, synthetic construct
APPSSFSKAKKEAVKIYLDYPTSFYCGCDITWKNKKKGIPELESCGYQVRKQEKRASRIEWEHVVPAWQFGHQRQCWKKKGRKNCTRNDKQFKSMEADLHNLVPAIGEVNGDRKNFRFSQWNGSKGAFYGQCAFKVDFKGRVAEPPAQSRGAIARTYLYMNNEYKFNLSKAQRQLMEAWNKQYPVSTWECTRDERIAKIQGNHNQFVYKACTK

SEQ ID NO: 28 - protein, 216 aa, synthetic construct
APPSSFSKAKKEAVKIYLDYPTSFYCGCDITWKNKKKGIPELESCGYQVRKQEKRASRIEWEHVVPAWQFGHQRQCWQKGGRKNCTRNDKQFKSMEADLHNLVPAIGEVNGDRSNFRFSQWNGSKGAFYGQCDMKIDFKNRRADPPEQSRGAIARTYLYMNQEYKMALSSQQRQLMEAWNRQYPISTWECERDRRIANIQDNHNSFVLQACKKAGY

SEQ ID NO: 29 - protein, 225 aa, synthetic construct
APPSSFSKAKRLAVEIYQDHPTSFYCGCAITWQGKKGLPDLASCGYEVRKQEKRANRIEWEHVVPAENFGRAFVEWREGHPQCVNSKGKAYKGRSCATKMNPTYRSMQADLHNLTPAVGEVNGDRSNYAFLPWNGNNGAFYGQCAFKVDFKGRVAEPPAQSRGAIARTYLYMNNEYKFNLSKAQRQLMEAWNKQYPVSTWECTRDERIAKIQGNHNQFVYKACTK

SEQ ID NO: 30 - protein, 216 aa, synthetic construct
APPSSFSKAKREAVKIYLDHPTSFYCGCDITWKDKKKGIPDLDSCGYQVRKQQKRASRIEWEHVVPAWQFGHQRQCWQDGGRKNCTRNDKIFKSMEADLHNLTPAIGEVNGDRSNYNFSQWNGMDGVSYGQCDIKVDFKNRRVDPPPRARGAIARTYLYMEQEYRFRLAKNQRQLMQAWHKSYPVSPWECERDRRIAKIQNKHNSFVLEACQQAGL

SEQ ID NO: 31 - protein, 216 aa, synthetic construct
APPSSFSKAKKLAVKIYLDHPTSFYCGCDITWKDKKKGIPDLESCGYEVRKQEKRASRIEWEHVVPAWQFGHQRQCWQDGGRKNCTKNDKNFKMMEADLHNLVPAIGEVNGDRSNFRFSQWNGSKGAFYGQCDMKIDFKNRRADPPEQSRGAIARTYLYMNQEYKMALSSQQRQLMEAWNRQYPISTWECERDRRIANIQDNHNSFVLQACNKAGY

SEQ ID NO: 32 - protein, 216 aa, synthetic construct
APPSSFSKAKKEAVKIYLDHPTSFYCGCDITWKDKKKGIPDLQSCGYDVRKQEKRASRIEWEHIVPAWQFGHQRQCWQDGGRKNCTRKDKQFKLMEADLHNLVPAIGEVNGDRSNFRFSQWNGNKGAFYGQCDMKIDFKNRRADPPEQSRGAIARTYLYMNQEYKMALSSQQRQLMEAWNRQYPVSTWECERDRRIANIQDNHNSFVLKACQKSGY

SEQ ID NO: 33 - protein, 250 aa, synthetic construct
QVPPLTELSPSISVHLLLGNPSGATPTKLTPDNYLMVKNQYALSYNNSKGTANWVAWQLNSSWLGNAERQDNFRPDKTLPAGWVRVTPSMYSGSGYARGHIAPSADRTKTTEDNAATFLMTNMMPQTPDNNRNTWGNLEDYCRELVSQGKELYIVAGPNGSLGKPLKGKVTVPKSTWKIVVVLDSPGSGLEGITANTRVIAVNIPNDPELNNDWRAYKVSVDELESLTGYDFLSNVSPNIQTSIESKVDN

SEQ ID NO: 34 - protein, 381 aa, synthetic construct
EDCVWDNDVDYPEYPPLILDSSFQLVLPVLEGDQRITSVQSGSKLILACPGRGISALGSEDAQATCLGGKLVEVDGKEWNIVELGCTKMASETIHRNLGQCGDQDLGIYEVIGFDLPTTGHFYELIRVCFDPANETTIFSENIVHGASIAAKDIDPGRPSFKTSTGFFSVSMISVYSQSSQLELMKNLLGDDELAATIIDPSEQFYFAKGHMAPDADFVTVVEQDATYYYINALPQWQAFNNGNWKYLEYDTRDLAEKHGTDLTVYSGGWGVLELEDINGNPVEIYLGLAQDKKVVPAPALTWKVIYEKDTNRAAAIVGINNPHITTAPEPLCTDICSSLTWLDFDFGDLVHGYTYCCSVADLRAAIPNVPDLGDVDILDE

SEQ ID NO: 35 - protein, 8 aa, synthetic construct
  VARIANT 5: note = Wherein X at position 5 is H or A
IEWEXVVP

SEQ ID NO: 36 - protein, 6 aa, synthetic construct
GGRKNC

SEQ ID NO: 37 - protein, 8 aa, synthetic construct
PAIGEVNG

SEQ ID NO: 38 - protein, 53 aa, synthetic construct
IEWEHVVPAWQFGHQRQCWQKGGRKNCTRNDKQFKSMEADLHNLVPAIGEVNG

SEQ ID NO: 39 - protein, 53 aa, synthetic construct
IEWEHVVPAWQFGHQLQCWQQGGRKNCTRTSPEFNQMEADLHNLTPAIGEVNG

SEQ ID NO: 40 - protein, 53 aa, synthetic construct
IEWEHVVPAWQFGHHRQCWQKGGRKNCSKNDQQFRLMEADLHNLTPAIGEVNG

SEQ ID NO: 41 - protein, 218 aa, Oceanimonas sp.
GEAMSFRQAKKVAPGIYNDNLKTFYCGCNIDTQGKKLVPDLAGCGYQVRKQQQRASRIEWEHVVPAWEFGHQRQCWQQGGRKNCTRKDELFRQMEGDLHNLVPAVGEVNGDRSNYRFSEWNGKPVQYGQCQMLVDFKGRKVQPPEQSRGAIARTYLYMQQQYRLKIARQQQKLFEAWNRQYPASPWECERDNRISRIQGNHNPFVQEQCKNYAYTPNP

SEQ ID NO: 42 - protein, 213 aa, Salmonella sp.
DGINNFSQAKAASVKVNADAPGSFYCGCQIRWQGKKGVVDLESCGYKVRKNENRARRIEWEHVVPAWQFGHQRQCWQDGGRKNCAKDPVYRKMESDMHNLQPAIGEVNGDRGNFMYSQWNGGEGQYGQCAMKVDFKAKLAEPPARARGAIARTYFYMRDQYQLKLSRQQTQLFNVWDKQYPVTAWECERDARIAKVQGNHNPYVQRACQARKS

SEQ ID NO: 43 - protein, 213 aa, Enterobacter sp.
DGINSFSQAKAAGVKVNADVPGDFYCGCKINWQGKKGIVDLESCGYKVRKNENRASRIEWEHVVPAWQFGHQRQCWQDGGRKNCAKDPVYRQMESDMHNLQPAVGEVNGDRGNFMYSQWNGGEGQYGQCGMKVDFKEKVAEPPARARGSIARTYFYMRDRYNLNLSRQQTQLFNAWNKQYPVTEWECQRDERIARVQGNHNPYVQRACQAQKS

SEQ ID NO: 44 - protein, 213 aa, Yokenella sp.
EGINSFSQAKAAGVKVNADVAGDFYCGCKINWQGKKGVVDLESCGYKVRKNENRASRIEWEHVVPAWQFGHQRQCWQDGGRKNCGKDPVYRQMESDMHNLQPAVGEVNGDRGNFMYSQWNGGEGQYGQCAMKVDFKGKVAEPPARARGAIARTYFYMRDRYQLALSRQQTQLFNAWDKQYPVSEWECERDERIAKYQGNHNPYVQRACQAQKS

SEQ ID NO: 45 - protein, 213 aa, Klebsiella sp.
AGINSFSQAKAAGVKVNADVPGDFYCGCKIDWQGKKGVIDLESCGYKVRKNENRASRVEWEHVVPAWQFGHQRQCWQEGGRKNCAKDPEYRKMESDMHNLQPAVGEVNGDRGNFMYSQWNGGEGQYGQCTMKVDFKDKIAEPPARARGAIARTYFYMRDRYQLNLSRQQTQLFTAWNKQYPVTAWECERDERIAKVQGNHNPYVQQACQAQKS

SEQ ID NO: 46 - protein, 213 aa, Escherichia coli
EGINSFSQAKAVAVKIHADAPGTFYCGCKIDWQGKKGVVDLQSCGYQVRKNENRASRVEWEHVVPAWQFGHQRQCWQDGGRKNCAKDPVYRKMESDMHNLQPSVGEVNGDRGNFMYSQWNGGEGQYGQCAMKVDFKEKVAEPPARARGAIARTYFYMRDQYNLTLSRQQTQLFNAWNKMYPVTDWECERDERIAKVQGNHNPYVQRACQARKS

SEQ ID NO: 47 - protein, 213 aa, Shigella sp.
EGINSFSQAKAAAVKVHADAPGTFYCGCKINWQGKKGVVDLQSCGYQVRKNENRASRVEWEHVVPAWQFGHQRQCWQDGGRKNCAKDPVYRKMESDMHNLQPSVGEVNGDRGNFMYSQWNGGEGQYGQCAMKVDFKEKAAEPPARARGAIARTYFYMRDQYNLTLSRQQTQLFNAWNKMYPVTDWECERDERIAKVQGNHNPYVQRACQARKS

SEQ ID NO: 48 - protein, 213 aa, Citrobacter sp.
EGINSFSQAKAAGVKVNADAPGDFYCGCKINWQGKKGVVDLESCGYKVRKNENRASRIEWEHVVPAWQFGHQRQCWQDGGRKNCAKDPVYRKMESDMHNLQPAVGEVNGDRANFMYSQWNGGEGQYGQCAMKVDFKEKVAEPPARARGAIARTYFYMRDQYSLTLSRQQTQLFNAWNKQYPVTDWECERDERIAKVQGNHNPYVQRACQAQKS

SEQ ID NO: 49 - protein, 214 aa, Cronobacter sp.
ASGIHSFSQAKAAGVKINADAPGDFYCGCPITWQGKKGIPDLKACGYQVRKNENRASRIEWEHVVPAWQFGHQRQCWQNGGRKNCDKDPVYREMETDLHNLQPAVGEVNGDRGNFLYSQWRGGEGQYGQCEMKVDFKNKQAEPPARARGAIARTYFYMRDKYQLNLSRAQTQLFEAWNKLYPVTPWECTRDERIAKVQGNHNPYVQQACQGQNR

SEQ ID NO: 50 - protein, 226 aa, Rahnella sp.
IGALVPLSAFSQSGNTINNFSQAKAAAVKINQGAPTFYCGCNIRWQGKKGTPDLQSCGYAVRKSELRASRIEWEHVVPAWQFGHQMQCWQDGGRKNCAKNADYRQVETDLHNLEPAIGEVNGDRNNFMYSQWNGGEGQYGRCEMKIDFKAKAAEPPARARGAIARTYFYMRDQYKLNLSRQQTQLFTAWDRQYPVTAWECERDNRIARVQGNHNPYVQQACAQRKS

SEQ ID NO: 51 - protein, 223 aa, Erwinia sp.
FPPLFCHALSQGNYQQNNFSQAKAWAAQIHHDAPGTFYCGCKIDWQGKKGVPDLTSCGYQVRKNSERASRIEWEHVVPAWSFGHQRQCWQDGGRKNCVKDPVYRRMESDLHNLQPAIGEVNGDRGNFMYGQWSGGEQQYGQCAMKVDFKNKLAEPPARARGAIARTWFYMRDQYQLSMSKQQTQLMTAWSKLYPVTPWECERDRRIARVQGNHNPYVQQACQR

SEQ ID NO: 52 - protein, 213 aa, Yersinia sp.
HGINNFSQAKAVAAKIHQDAPGSFYCGCQIDWQGKKGIPDLNSCGYQPRKNAARAARIEWEHVVPAWQFGHQRQCWQQGGRKNCAKDPVYRQIETDLHNLQPAIGEVNGDRNNFMYSQWNGGSGQYGQCAMKVDFKNKLAEPPVRARGAIARTYFYMRDQYQLRLSSQQSKLFGVWDRQYPVTDWECLRDERIAKTQGNHNPYVQRACQRPKS

SEQ ID NO: 53 - protein, 213 aa, Serratia sp.
HGINNFSQAKAAAAKINQDAPGSFYCGCKINWHGKKGLPDLNACGYQPRKNAQRAGRIEWEHVVPAWQFGHQLQCWQDGGRKNCNRDPVYRQIETDLHNLQPAIGEVNGDRNNFMYSQWRGGEGQYGQCPMKVDFKHKQAEPPARARGAIARTYFYMRDRYHLRLSRQQTQLFEVWNRQYPVSQWECQREARIAKVQGNRNPYIQQACQRQKG

SEQ ID NO: 54 - protein, 213 aa, Pseudomonas synxantha
AQAQAPRTFSEAKKVAWGLYAPQSTEFYCGCKYTGKRVDLAGCGYVPRKSAKRASRIEWEHIVPAWQIGHLRQCWQNGGRKNCTKSDPVYKRAEADLHNLVPSIGEVNGDRSNFSFGWVPEQKGQYGSCLTQVDFKAKKVMPRPSIRGMIARTYFYMSKQYNLRLSRQDQQLYQAWDKTYPPQIWERQRNQQVACVMGRGNEFVGPVDLKACK

SEQ ID NO: 55 - protein, 213 aa, Aliivibrio fischeri
APPSSFSKAKKEAVKIYLDHPTSFYCGCDITWKDKKKGIPDLQSCGYNVRKQEKRASRIEWEHVVPAWQFGHQRQCWQDGGRKNCTRKDKQFKLMEADLHNLVPAIGEVNGDRSNFRFSQWNGNKGAYYGQCAFKVDFKGRVAEPPAQSRGAIARTYLYMNQEYRFNLSKSQRQLMNAWDKQYPVSEWECERDKRIAKIQGNHNQFVYKACRK

SEQ ID NO: 56 - protein, 213 aa, Aliivibrio wodanis
APPSSFSKAKKLAVKIYLDHPTSFYCGCDITWKDKKKGIPDLESCGYEVRKQEKRASRIEWEHVVPAWQFGHQRQCWQDGGRKNCTKNDKNFKMMEADLHNLVPAIGEVNGDRSNFRFSQWNGSKGANYGQCAFKVDFKGRVAEPPAQSRGAIARTYMYMNKEYRFNLSKAQRQLMEAWDKQYPVSAWECERDQRIAKIQGNHNQFVFKACTK

SEQ ID NO: 57 - protein, 212 aa, Vibrio splendidus
APPSSFSKAKKEAVKIYLDHPTSFYCGCDITWKDKKKGIPDLDGCGYQVRKQQKRASRIEWEHVVPAWQFGHQRQCWQDGGRKNCTRNDKVFKSMEADLHNLTPAIGEVNGDRSNYNFSQWNSMDGVSYGQCEMQVNFKQRKVMPPDRAKGSIARTYLYMSQEYGFKLSKQQTNLMMAWNKQFPVNEWECTRDERIFAIQGNHNPFVYQACK

SEQ ID NO: 58 - protein, 212 aa, Vibrio harveyi
APPSSFSAAKREAVKIYADHPTSFYCGCDIKWQGKKGIPDLASCGYQVRKQEKRASRIEWEHVVPAWQFGHQRQCWQNGGRKNCTRNDNVFKSMEADLHNLTPAIGEVNGDRSNYNFSQWNGMDGVSYGRCEMQVNFKQRKVMPPDRARGSIARTYLYMSKEYGFKLSKQQTQLMSAWNKSYPVDKWECERDERIAKIQGNHNPFVQEACRA

SEQ ID NO: 59 - protein, 212 aa, Vibrio rotiferianus
APPSSFSAAKREAVKIYADHPTSFYCGCDIKWQGKKGVPDLASCGYQVRKQEKRASRIEWEHVVPAWQFGHQRQCWQNGGRKNCTRNDKVFKSMEADLHNLTPAIGEVNGDRSNYNFSQWNGMDGVSYGRCEMQVNFKQRKVMPPDRARGSIARTYLYMSKEYGFKLSKQQTQLMSAWNKTYPVDKWECERDERIAKIQGNHNPFVQEACRA

SEQ ID NO: 60 - protein, 213 aa, Vibrio tubiashii
APPSSFSKAKKEAVKIYADHPTSFYCGCNISWQGRKGIPDLESCGYQVRKQQKRASRIEWEHVVPAWQFGHQRQCWQNGGRKNCTKNDKAFRMMEADLHNLTPAIGEVNGDRSNYNFSQWNGIDGVSYGRCEMQVNFKHRKVMPPDRAKGSIARTYLYMSQEYGFRLSKQQTQLMNAWNKQFPVDHWECEREQRIFKVQGNHNPFVHQACQAL

SEQ ID NO: 61 - protein, 204 aa, Vibrio sinaloensis
APPSSFSKAKKEAIKIYADHPSSFYCGCDITWQGRKGTPDLNSCGYQVRKQEKRASRIEWEHVVPAWQFGHQRQCWQNGGRKNCSKNDNVFRSMEADLHNLTPAIGEVNGDRSNYNFSQWNGVDGVSYGRCEMQVNFKQRKVMPPDRAKGSIARTYLYMSKEYGFKLSKQQTQLMTAWNKQFPVDEWECERDKRIFKVQGNHNP

SEQ ID NO: 62 - protein, 213 aa, Vibrio vulnificus
APPSSFSAAKQQAVKIYQDHPISFYCGCDIEWQGKKGIPNLETCGYQVRKQQTRASRIEWEHVVPAWQFGHQRQCWQKGGRKNCSKNDQQFRLMEADLHNLTPAIGEVNGDRSNFNFSQWNGMDGVSYGRCEMQVNFKQRKVMPPDRARGSIARTYLYMSQEYGFQLSKQQQQLMQAWNKSYPVDEWECTRDDRIAKIQGNHNPFVQQSCTVR

SEQ ID NO: 63 - protein, 211 aa, Vibrio furnissii
APASFSQAKREAVKIYQDHPVTFYCGCDIQWQGKKGTPDLKGCGYQVRKQEKRASRIEWEHVVPAWQFGHQLQCWQQGGRKQCSRHDTAFKRMEADLHNLTPAIGEVNGDRSNLNFSQWHGIDGATYGQCEIQVNFQQRKVMPPERARGAIARTYLYMSQEYGFRLSKSQTQLMQVWNRQYPVDSWECERDQRIFKVQGNHNPFVRQQCSS

SEQ ID NO: 64 - protein, 212 aa, Vibrio anguillarum
APPASFSQAKKEALKIYHDHPVSFYCGCDIAWQGKKGTPDLQACGYQVRKQQTRASRIEWEHVVPAWQFGHQRQCWQQGGRKNCTKNDTIFRSMEADLHNLTPAIGEVNGDRSNYNFSQWNGVEGESYGRCEMQVDFKQRKVMPPDRARGSIARTYLYMSQNYGFQLSKSQTQLMQAWNRQYPADEWECKRDQRIAKVQGNHNPFVQQQCRS

SEQ ID NO: 65 - protein, 245 aa, synthetic construct
DTLESIDNCAVGCPTGGSSNVSIVRHAYTLNNNSTTKFANWVAYHITKDTLASGKTRRWKTDPALNPADTLAPADYKGANAALKVDRGHQAPLASLAGVSDWESLNYLSNITPQKSDLNQGAWKRLEDQERKLIDRADISSVYTVTGPLYERDMGKLPGTQKAHTIPSAYWKVIFINNSPAVNHYAAFLFDQNTPKKADFCQFRVTVDEIEKRTGLIIWAGLPDDVQASLKSKPGVLPELMGCKN

SEQ ID NO: 66 - protein, 245 aa, synthetic construct
DTLESIDNCAVGCPTGGSSNVSIVRHAYTLNNNSTTKFANWVAYHITKDTLASGKTRNWKTDPALNPADTLAPADYRGANAALKVDRGHQAPLASLAGVSDWESLNYLSNITPQKSDLNQGAWKRLEDQERKLIDRADISSVYTVTGPLYERDMGKLPGTQKAHTIPSAYWKVIFINNSPAVNHYAAFLFDQNTPKKADFCQFRVTVDEIEKRTGLIIWAGLPDDVQASLKSKPGVLPELMGCKN

SEQ ID NO: 67 - protein, 118 aa, Bacillus licheniformis
YSPQHAEGAARYDDILYFPASRYPETGAHISDAIKAGHSDVCTIERSGADKRRQESLKGIPTKPGFDRDEWPMAMCEEGGKGASVRYVSSSDNRGAGSWVGNRLSGFADGTRILFIVQ

SEQ ID NO: 68 - protein, 381 aa, Pandalus borealis
EDCVWDNDVDYPEYPPLILDSSFQLVLPVLEGDQRITSVQSGSELILACPGREISALGSEDAQATCLGGKLVEVDGKEWNIVELGCTKMASETIHRNLGQCGDQDLGIYEVIGFDLPTTGHFYELIRVCFDPANETTIFSENIVHGASIAAKDIDPGRPSFKTSTGFFSVSMISVYSQRNQLELMKNLLGDDELAATIIDPSKQFYFAKGHMAPDADFVTVVEQDATYYYINALPQWQAFNNGNWKYLEYDTRDLAEKHGTDLTVYSGGWGVLELEDINGNPVEIYLGLAQDKKVVPAPALTWKVIYEKDTNRAAAIVGINNPHITTAPEPLCTDICSSLTWLDFDFGDLVHGYTYCCSVADLRAAIPNVPDLGDVDILDE